European Patent Specification EP 4 110 940 B1, published March 27, 2024. Title: METHOD AND APPARATUS FOR ENZYMATIC SYNTHESIS OF POLYNUCLEOTIDES. Applicant: DNA SCRIPT. The sequence listing filed with the application follows.

SEQUENCE LISTING (30 sequences)

SEQ ID NO: 1 - DNA, 21 bp, ARTIFICIAL SEQUENCE
  nucleotide
gtttcctaagttgcatttgcg

SEQ ID NO: 2 - protein, 381 aa, ARTIFICIAL SEQUENCE
  truncated mouse TdT
NSSPSPVPGSQNVPAPAVKKISQYACQRRTTLNNYNQLFTDALDILAENDELRENEGSCLAFMRASSVLKSLPFPITSMKDTEGIPCLGDKVKSIIEGIIEDGESSEAKAVLNDERYKSFKLFTSVFGVGLKTAEKWFRMGFRTLSKIQSDKSLRFTQMQKAGFLYYEDLVSCVNRPEAEAVSMLVKEAVVTFLPDALVTMTGGFRRGKMTGHDVDFLITSPEATEDEEQQLLHKVTDFWKQQGLLLYCDILESTFEKFKQPSRKVDALDHFQKCFLILKLDHGRVHSEKSGQQEGKGWKAIRVDLVMCPYDRRAFALLGWTGSRQFERDLRRYATHERKMMLDNHALYDRTKRVFLEAESEEEIFAHLGLDYIEPWERNA

SEQ ID NO: 3 - protein, 380 aa, BOVINE
DYSATPNPGFQKTPPLAVKKISQYACQRKTTLNNYNHIFTDAFEILAENSEFKENEVSYVTFMRAASVLKSLPFTIISMKDTEGIPCLGDKVKCIIEEIIEDGESSEVKAVLNDERYQSFKLFTSVFGVGLKTSEKWFRMGFRSLSKIMSDKTLKFTKMQKAGFLYYEDLVSCVTRAEAEAVGVLVKEAVWAFLPDAFVTMTGGFRRGKKIGHDVDFLITSPGSAEDEEQLLPKVINLWEKKGLLLYYDLVESTFEKFKLPSRQVDTLDHFQKCFLILKLHHQRVDSSKSNQQEGKTWKAIRVDLVMCPYENRAFALLGWTGSRQFERDIRRYATHERKMMLDNHALYDKTKRVFLKAESEEEIFAHLGLDYIEPWERNA

SEQ ID NO: 4 - protein, 380 aa, HUMAN
DYSDSTNPGPPKTPPIAVQKISQYACQRRTTLNNCNQIFTDAFDILAENCEFRENEDSCVTFMRAASVLKSLPFTIISMKDTEGIPCLGSKVKGIIEEIIEDGESSEVKAVLNDERYQSFKLFTSVFGVGLKTSEKWFRMGFRTLSKVRSDKSLKFTRMQKAGFLYYEDLVSCVTRAEAEAVSVLVKEAVWAFLPDAFVTMTGGFRRGKKMGHDVDFLITSPGSTEDEEQLLQKVMNLWEKKGLLLYYDLVESTFEKLRLPSRKVDALDHFQKCFLIFKLPRQRVDSDQSSWQEGKTWKAIRVDLVLCPYERRAFALLGWTGSRQFERDLRRYATHERKMILDNHALYDKTKRIFLKAESEEEIFAHLGLDYIEPWERNA

SEQ ID NO: 5 - protein, 376 aa, CHICKEN
QYPTLKTPESEVSSFTASKVSQYSCQRKTTLNNCNKKFTDAFEIMAENYEFKENEIFCLEFLRAASVLKSLPFPVTRMKDIQGLPCMGDRVRDVIEEIIEEGESSRAKDVLNDERYKSFKEFTSVFGVGVKTSEKWFRMGLRTVEEVKADKTLKLSKMQRAGFLYYEDLVSCVSKAEADAVSSIVKNTVCTFLPDALVTITGGFRRGKKIGHDIDFLITSPGQREDDELLHKGLLLYCDIIESTFVKEQIPSRHVDAMDHFQKCFAILKLYQPRVDNSSYNMSKKCDMAEVKDWKAIRVDLVITPFEQYAYALLGWTGSRQFGRDLRRYATHERKMMLDNHALYDKRKRVFLKAGSEEEIFAHLGLDYVEPWERNA

SEQ ID NO: 6 - protein, 387 aa, POSSUM
SANPDPTAGTLNILPPTTKTISQYACQRRTTINNHNQRFTDAFEILAKNYEFKENDDTCLTFMRAISVLKCLPFEVVSLKDTEGLPWIGDEVKGIMEEIIEDGESLEVQAVLNDERYQSFKLFTSVFGVGLKTADKWYRMGFRTLNKIRSDKTLKLTKMQKAGLCYYEDLIDCVSKAEADAVSLLVQDAVWTFLPDALVTITGGFRRGKEFGHDVDFLITSPGAEKEQEDQLLQKVTNLWKKQGLLLYCDLIESTFEDLKLPSRKIDALDHFQKCFLILKLYHHKEDKRKWEMPTGSNESEAKSWKAIRVDLVVCPYDRYAFALLGWSGSRQFERDLRRYATHEKKMMLDNHALYDKTKKIFLKAKSEEEIFAHLGLEYIQPSERNA

SEQ ID NO: 7 - protein, 381 aa, SHREW
DCPASHDSSPQKTESAAVQKISQYACQRRTTLNNHNHIFTDAFEILAENCEFRENEGSYVTYMRAASVLKSLPFSIISMKDTEGIPCLADKVKCVIEEIIEDGESSEVKAVLNDERYKSFKLFTSVFGVGLKTAEKWFRLGFRTLSGIMNDKTLKLTHMQKAGFLYYEDLVSCVTRAEAEAVGVLVKEAVWAFLPDAIVTMTGGFRRGKKVGHDVDFLITSPEATEEQEQQLLHKVITFWEKEGLLLYCDLYESTFEKLKMPSRKVDALDHFQKCFLILKLHRECVDDGTSSQLQGKTWKAIRVDLVVCPYECRAFALLGWTGSPQFERDLRRYATHERKMMLDNHALYDKTKRKFLSADSEEDIFAHLGLDYIEPWERNA

SEQ ID NO: 8 - protein, 387 aa, PYTHON
EKYQLPEDEDRSVTSDLDRDSISEYACQRRTTLKNYNQKFTDAFEILAENYEFNENKGFCTAFRRAASVLKCLPFTIVQVHDIEGVPWMGKQVKGIIEDIIEEGESSKVKAVLDNENYRSVKLFTSVFGVGLKTSDKWYRMGLRTLEEVKRDKNLKLTRMQKAGFLHYDDLTSCVSKAEADAASLIVQDVVWKIVPNAIVTIAGGFRRGKQTGHDVDFLITVPGSKQEEEELLHTVIDIWKKQELLLYYDLIESTFEDTKLPSRKVDALDHFQKCFAILKVHKEREDKGNSIRSKAFSEEEIKDWKAIRVDLVVVPFEQYAFALLGWTGSTQFERDLRRYATHEKKMMLDNHALYDKTKKIFLNAASEEEIFAHLGLDYLEPWERNA

SEQ ID NO: 9 - protein, 381 aa, DOG
DYTASPNPELQKTLPVAVKKISQYACQRRTTLNNYNNVFTDAFEVLAENYEFRENEVFSLTFMRAASVLKSLPFTIISMKDTEGIPCLGDQVKCIIEEIIEDGESSEVKAVLNDERYQSFKLFTSVFGVGLKTSEKWFRMGFRTLSKIKSDKSLKFTPMQKAGFLYYEDLVSCVTRAEAEAVGVLVKEAVGAFLPDAFVTMTGGFRRGKKMGHDVDFLITSPGSTDEDEEQLLPKVINLWERKGLLLYCDLVESTFEKLKLPSRKVDALDHFQKCFLILKLHHQRVDGGKCSQQEGKTWKAIRVDLVMCPYERRAFALLGWTGSRQFERDLRRYASHERKMILDNHALYDKTKKIFLKAESEEEIFAHLGLDYIEPWERNA

SEQ ID NO: 10 - protein, 382 aa, TRUNC MOLE
GDCPASHDSSPQKTESAAVQKISQYACQRRTTLNNHNHIFTDAFEILAENCEFRENEGSYVTYMRAASVLKSLPFSIISMKDTEGIPCLADKVKCVIEEIIEDGESSEVKAVLNDERYKSFKLFTSVFGVGLKTAEKWFRLGFRTLSGIMNDKTLKLTHMQKAGFLYYEDLVSCVTRAEAEAVGVLVKEAVWAFLPDAIVTMTGGFRRGKKVGHDVDFLITSPEATEEQEQQLLHKVITFWEKEGLLLYCDLYESTFEKLKMPSRKVDALDHFQKCFLILKLHRECVDDGTSSQLQGKTWKAIRVDLVVCPYECRAFALLGWTGSPQFERDLRRYATHERKMMLDNHALYDKTKRKFLSADSEEDIFAHLGLDYIEPWERNA

SEQ ID NO: 11 - protein, 379 aa, PIKA TRUNK
EYSANPSPGPQATPAVYKISQYACQRRTTLNNHNHIFTDAFEILAENYEFKENEGCYVTYMRAASVLKSLPFTIVSMKDTEGIPCLEDKVKSIMEEIIEEGESSEVKAVLSDERYQCFKLFTSVFGVGLKTSEKWFRMGFRSLSNIRLDKSLKFTQMQKAGFRYYEDIVSCVTRAEAEAVDVLVNEAVRAFLPDAFITMTGGFRRGKKIGHDVDFLITSPELTEEDEQQLLHKVMNLWEKKGLLLYHDLVESTFEKLKQPSRKVDALDHFQKCFLIFKLYHERVGGDRCRQPEGKDWKAIRVDLVMCPYECHAFALLGWTGSRQFERDLRRYASHERKMILDNHALYDKTKRVFLQAENEEEIFAHLGLDYIEPWERNA

SEQ ID NO: 12 - protein, 384 aa, TRUNC HEDGEHOG
DASFGSNPGSQNTPPLAIKKISQYACQRRTSLNNCNHIFTDALDILAENHEFRENEVSCVAFMRAASVLKSLPFTIISMKDTKGIPCLGDKAKCVIEEIIEDGESSEVKAILNDERYQSFKLFTSVFGVGLKTSEKWFRMGFRTLNKIMSDKTLKLTRMQKAGFLYYEDLVSCVAKAEADAVSVLVQEAVWAFLPDAMVTMTGGFRRGKKLGHDVDFLITSPGATEEEEQQLLPKVINFWERKGLLLYHDLVESTFEKLKLPSRKVDALDHFQKCFLILKLHLQHVNGVGNSKTGQQEGKNWKAIRVDLVMCPYERRAFALLGWTGSRQFERDLRRFATHERKMMLDNHALYDKTKRIFLKAESEEEIFAHLGLDYIDPWERNA

SEQ ID NO: 13 - protein, 381 aa, TREE SHREW
DHSTSPSPGPQKTPALAVQKISQYACQRRTTLNNCNRVFTDAFETLAENYEFRENEDSSVIFLRAASVLRSLPFTITSMRDTEGLPCLGDKVKCVIEEIIEDGESSEVNAVLNDERYKSFKLFTSVFGVGLKTSEKWFRMGFRTLSRVRSDKSLHLTRMQQAGFLYYEDLASCVTRAEAEAVGVLVKEAVGAFLPDALVTITGGFRRGKKTGHDVDFLITSPGSTEEKEEELLQKVLNLWEKKGLLLYYDLVESTFEKLKTPSRKVDALDHFPKCFLILKLHHQRVDGDKPSQQEGKSWKAIRVDLVMCPYERHAFALLGWTGSRQFERDLRRYATHERKMMLDNHALYDKTKRVFLKAESEEDIFAHLGLDYIEPWERNA

SEQ ID NO: 14 - protein, 394 aa, PLATYPUS
LTNSAPINCMTETPSLATKQVSQYACERRTTLNNCNQKFTDAFEILAKDFEFRENEGICLAFMRAISVLKCLPFTIVRMKDIEGVPWLGDQVKSIIEEIIEDGESSSVKAVLNDERYRSFQLFNSVFEVGLTDNGENGIARGFQTLNEVITDENISLTKTTLSTSLWNYLPGFLYYEDLVSCVAKEEADAVYLIVKEAVRAFLPEALVTLTGGFRRGKKIGHDVDFLISDPESGQDEQLLPNIIKLWEKQELLLYYDLVESTFEKTKIPSRKVDAMDHFQKCFLILKLHHQKVDSGRYKPPPESKNHEAKNWKAIRVDLVMCPFEQYAYALLGWTGSRQFERDLRRYATHEKKMMLDNHALYDKTKKIFLKAESEEDIFTHLGLDYIEPWERNA

SEQ ID NO: 15 - protein, 384 aa, JERBOA
SSELELLDVSWLIECMGAGKPVEMTGRHQLVKQTFCLPGFILQDAFDILAENCEFRENEASCVEFMRAASVLKSLPFPIISVKDTEGIPWLGGKVKCVIEEIIEDGESSEVKALLNDERYKSFKLFTSVFGVGLKTAERWFRMGFRTLSTVKLDKSLTFTRMQKAGFLHYEDLVSCVTRAEAEAVSVLVQQAVVAFLPDALVSMTGGFRRGKKIGHDVDFLITSPEATEEEEQQLLHKVTNFWEQKGLLLYCDHVESTFEKCKLPSRKVDALDHFQKCFLILKLYRERVDSVKSSQQEGKGWKAIRVDLVMCPYECRAFALLGWTGSRQFERDLRRYATHERKMRLDNHALYDKTKRVFLKAESEEEIFAHLGLEYIEPLERNA

SEQ ID NO: 16 - protein, 362 aa, Truncated mouse
KISQYACQRRTTLNNYNELFTRALDILAENDEFRENEESRDAFRRASSVLKSLPFPITSMKDTEGIPCLGDKVKRIIEEIIEDGESSEVKAVLNDERYKAFKLFTSVFGVGRKTAEKWFRMGFRTLEKIRSDKSLRFTQMQKAGFLYYEDLAERVNRPEAEAIRMLVKEAVVTFLPDALVTMTGGFRLGKMTGHDVDFLITSPEATEDEEQQLLHKVTDFWKQQGLLLYCDILESTFEKFKQPSRTVDALDHFQKCFLILKLDHPRVHSVKSGQQEGKGWKAIRVDLVMCPYDRRAFALLGWTGSPQFNRDLRRYATHERKMMLDNHALYDKTKRVFLEAESEEEIFAHLGLDYIEPWERNA

SEQ ID NO: 17 - protein, 361 aa, Artificial Sequence
  bovine-mouse chimera (M57 without His tag & linker)
KISQYACQRRTTLNNYNELFTRALDILAENDEFRENEESRDAFRRASSVLKSLPFPITSMKDTEGIPCLGDKVKRIIEEIIEDGESSEVKAVLNDERYKAFKLFTSVFGVGRKTAEKWFRMGFRTLEKIRSDKSLRFTQMQKAGFLYYEDLVSGVTRAEAEAVGVLVKEAVWAFLPDAFVTMTGGFRLGKKIGHDVDFLITSPGSAEDEEQLLPKVINLWEKKGLLLYYDLVESTFEKFKLPSRQVDTLDHFQKCFLILKLHHQRVDSSKSNQQEGKTWKAIRVDLVMCPYENRAFALLGWTGSPQFNRDLRRYATHERKMMLDNHALYDKTKRVFLEAESEEEIFAHLGLDYIEPWERNA

SEQ ID NO: 18 - protein, 361 aa, Artificial Sequence
  bovine-mouse chimera (M59 without His Tag and linker)
KISQYACQRRTTLNNYNELFTRALDILAENDEFRENEESRDAFRRASSVLKSLPFPITSMKDTEGIPCLGDKVKRIIEEIIEDGESSEVKAVLNDERYKAFKLFTSVFGVGRKTAEKWFRMGFRTLEKIRSDKSLRFTQMQKAGFLYYEDLAERVNRPEAEAIRMLVKEAVVTFLPDALVTMTGGFRLGKMTGHDVDFLITSPGSAEDEEQLLPKVINLWEKKGLLLYYDLVESTFEKFKLPSRQVDTLDHFQKCFLILKLHHQRVDSSKSNQQEGKTWKAIRVDLVMCPYENRAFALLGWTGSPQFNRDLRRYATHERKMMLDNHALYDKTKRVFLEAESEEEIFAHLGLDYIEPWERNA

SEQ ID NO: 19 - protein, 361 aa, mouse; identical to SEQ ID NO: 18

SEQ ID NO: 20 - protein, 361 aa, Artificial Sequence
  M54
KISQYACQRKTTLNNYNEIFTRAFEILAENSEFKENEESYVTFRRAASVLKSLPFTIISMKDTEGIPCLGDKVKRIIEEIIEDGESSEVKAVLNDERYQAFKLFTSVFGVGRKTSEKWFRMGFRSLEKIRSDKTLKFTKMQKAGFLYYEDLVSGVTRAEAEAVGVLVKEAVWAFLPDAFVTMTGGFRLGKKIGHDVDFLITSPGSAEDEEQLLPKVINLWEKKGLLLYYDLVESTFEKFKLPSRQVDTLDHFQKCFLILKLHHQRVDSSKSNQQEGKTWKAIRVDLVMCPYENRAFALLGWTGSAFFNRDIRRYATHERKMMLDNHALYDKTKRVFLKAESEEEIFAHLGLDYIEPRERNA

SEQ ID NO: 21 - protein, 362 aa, Artificial Sequence
  M77 without His tag
KKISEYACQRRTTLNNYNELFTRALDILAENDEFRENEESRDAFRRASSVLKSLPFPITSMKDTEGIPCLGDKVKRIIEEIIEDGESSEVKAVLNDERYKAFKLFTSVFGVGRKTAEKWFRMGFRTLEKIRSDKSLRFTQMQKAGFLYYEDLVSGVTRAEAEAVGVLVKEAVWAFLPDAFVTMTGGFRLGKKIGHDVDFLITSPGSAEDEEQLLPKVINLWEKKGLLLYYDLVESTFEKFKLPSRQVDTLDHFQKCFLILKLHHQRVDSSKSNQQEGKTWKAIRVDLVMCPYENRAFALLGWTGSPQFNRDLRRYATHERKMMLDNHALYDKTKRVFLEAESEEEIFAHLGLDYIEPWERNA

SEQ ID NO: 22 - protein, 377 aa, Artificial Sequence
  M77 with His tag
MASSHHHHHHSSGSEKKISEYACQRRTTLNNYNELFTRALDILAENDEFRENEESRDAFRRASSVLKSLPFPITSMKDTEGIPCLGDKVKRIIEEIIEDGESSEVKAVLNDERYKAFKLFTSVFGVGRKTAEKWFRMGFRTLEKIRSDKSLRFTQMQKAGFLYYEDLVSGVTRAEAEAVGVLVKEAVWAFLPDAFVTMTGGFRLGKKIGHDVDFLITSPGSAEDEEQLLPKVINLWEKKGLLLYYDLVESTFEKFKLPSRQVDTLDHFQKCFLILKLHHQRVDSSKSNQQEGKTWKAIRVDLVMCPYENRAFALLGWTGSPQFNRDLRRYATHERKMMLDNHALYDKTKRVFLEAESEEEIFAHLGLDYIEPWERNA

SEQ ID NO: 23 - protein, 361 aa, Artificial Sequence
  C1-40 without His tag
KISEYACQRRTTLNNYNELFTRALDILAENDEFRENEESRDAFRRASSVLKSLPFPITSMKDTEGIPCLGDKVKRIIEEIIEDGESSEVKAVLNDERYKAFKLFTSVFGVGRKTAEKWFRMGFRTLEKIRSDKSLRFTQMQKAGFLYYEDLVSGVTRAEAEAVGVLVKEAVWAFLPDAFVTMTGGFRLGKKIGHDVDFLITSPGSAEDEEQLLPKVINLWEKKGLLLYYDLVESTFEKFKLPSRQVDTLDHFQKCFLILKLHHQRVDSSKSNQQEGKTWKAIRVDLVMCPYENRAFALLGWTGSPQFNRDLRRYATHERKMMLDNHALYDKTKRVFLEAESEEEIFAHLGLDYIEPWERNA

SEQ ID NO: 24 - protein, 376 aa, Artificial Sequence
  C1-40 with His tag
MASSHHHHHHSSGSEKISEYACQRRTTLNNYNELFTRALDILAENDEFRENEESRDAFRRASSVLKSLPFPITSMKDTEGIPCLGDKVKRIIEEIIEDGESSEVKAVLNDERYKAFKLFTSVFGVGRKTAEKWFRMGFRTLEKIRSDKSLRFTQMQKAGFLYYEDLVSGVTRAEAEAVGVLVKEAVWAFLPDAFVTMTGGFRLGKKIGHDVDFLITSPGSAEDEEQLLPKVINLWEKKGLLLYYDLVESTFEKFKLPSRQVDTLDHFQKCFLILKLHHQRVDSSKSNQQEGKTWKAIRVDLVMCPYENRAFALLGWTGSPQFNRDLRRYATHERKMMLDNHALYDKTKRVFLEAESEEEIFAHLGLDYIEPWERNA

SEQ ID NO: 25 - protein, 363 aa, Artificial Sequence
  A2-20 without His tag
VTTVSEYACQRRTTLNNYNELFTRALDILAENDEFRENEESRDAFRRASSVLKSLPFPITSMKDTEGIPCLGDKVKRIIEEIIEDGESSEVKAVLNDERYKAFKLFTSVFGVGRKTAEKWFRMGFRTLEKIRSDKSLRFTQMQKAGFLYYEDLVSGVTRAEAEAVGVLVKEAVWAFLPDAFVTMTGGFRLGKKIGHDVDFLITSPGSAEDEEQLLPKVINLWEKKGLLLYYDLVESTFEKFKLPSRQVDTLDHFQKCFLILKLHHQRVDSSKSNQQEGKTWKAIRVDLVMCPYENRAFALLGWTGSPQFNRDLRRYATHERKMMLDNHALYDKTKRVFLEAESEEEIFAHLGLDYIEPWERNA

SEQ ID NO: 26 - protein, 379 aa, Artificial Sequence
  A2-20 with His tag
MASSHHHHHHSSGSENVTTVSEYACQRRTTLNNYNELFTRALDILAENDEFRENEESRDAFRRASSVLKSLPFPITSMKDTEGIPCLGDKVKRIIEEIIEDGESSEVKAVLNDERYKAFKLFTSVFGVGRKTAEKWFRMGFRTLEKIRSDKSLRFTQMQKAGFLYYEDLVSGVTRAEAEAVGVLVKEAVWAFLPDAFVTMTGGFRLGKKIGHDVDFLITSPGSAEDEEQLLPKVINLWEKKGLLLYYDLVESTFEKFKLPSRQVDTLDHFQKCFLILKLHHQRVDSSKSNQQEGKTWKAIRVDLVMCPYENRAFALLGWTGSPQFNRDLRRYATHERKMMLDNHALYDKTKRVFLEAESEEEIFAHLGLDYIEPWERNA

SEQ ID NO: 27 - protein, 363 aa, Artificial Sequence
  ii-ell-40 without His tag
VATVSEYACQRRTTLNNYNELFTRALDILAENDEFRENEESRDAFRRASSVLKSLPFPITSMKDTEGIPCLGDKVKRIIEEIIEDGESSEVKAVLNDERYKAFKLFTSVFGVGRKTAEKWFRMGFRTLEKIRSDKSLRFTQMQKAGFLYYEDLVSGVTRAEAEAVGVLVKEAVWAFLPDAFVTMTGGFRLGKKIGHDVDFLITSPGSAEDEEQLLPKVINLWEKKGLLLYYDLVESTFEKFKLPSRQVDTLDHFQKCFLILKLHHQRVDSSKSNQQEGKTWKAIRVDLVMCPYENRAFALLGWTGSPQFNRDLRRYATHERKMMLDNHALYDKTKRVFLEAESEEEIFAHLGLDYIEPWERNA

SEQ ID NO: 28 - protein, 379 aa, Artificial Sequence
  ii-ell-40 with His tag
MASSHHHHHHSSGSENVATVSEYACQRRTTLNNYNELFTRALDILAENDEFRENEESRDAFRRASSVLKSLPFPITSMKDTEGIPCLGDKVKRIIEEIIEDGESSEVKAVLNDERYKAFKLFTSVFGVGRKTAEKWFRMGFRTLEKIRSDKSLRFTQMQKAGFLYYEDLVSGVTRAEAEAVGVLVKEAVWAFLPDAFVTMTGGFRLGKKIGHDVDFLITSPGSAEDEEQLLPKVINLWEKKGLLLYYDLVESTFEKFKLPSRQVDTLDHFQKCFLILKLHHQRVDSSKSNQQEGKTWKAIRVDLVMCPYENRAFALLGWTGSPQFNRDLRRYATHERKMMLDNHALYDKTKRVFLEAESEEEIFAHLGLDYIEPWERNA

SEQ ID NO: 29 - protein, 363 aa, Artificial Sequence; identical to SEQ ID NO: 27
  9-40 without His tag

SEQ ID NO: 30 - protein, 379 aa, Artificial Sequence; identical to SEQ ID NO: 28
  9-40 with His tag